European Patent Application EP 4 454 650 A1, published October 30, 2024. Title: Antiviral composition comprising nucleoside analogues derived from nucleic acid or pharmaceutically acceptable salt thereof. Applicant: CJ CheilJedang Corporation. The sequence listing filed with the application follows.

SEQUENCE LISTING (12 sequences)

SEQ ID NO: 1 - DNA, 20 bp, synthetic construct
  misc_feature 1..20: note = PCV2 specific forward primer
  source 1..20: mol_type = other DNA
aggagggcgttctgactgtg

SEQ ID NO: 2 - DNA, 20 bp, synthetic construct
  misc_feature 1..20: note = PCV2 specific reverse primer
  source 1..20: mol_type = other DNA
accgctaccgttggagaagg

SEQ ID NO: 3 - DNA, 25 bp, synthetic construct
  misc_feature 1..25: note = SIV specific forward primer
  source 1..25: mol_type = other DNA
gatggtagatggatggtacggttat

SEQ ID NO: 4 - DNA, 26 bp, synthetic construct
  misc_feature 1..26: note = SIV specific reverse primer
  source 1..26: mol_type = other DNA
ttgttagtaatctcgtcaatggcatt

SEQ ID NO: 5 - DNA, 22 bp, synthetic construct
  misc_feature 1..22: note = IBV specific forward primer
  source 1..22: mol_type = other DNA
atgctcaaccttgtccctagca

SEQ ID NO: 6 - DNA, 21 bp, synthetic construct
  misc_feature 1..21: note = IBV specific reverse primer
  source 1..21: mol_type = other DNA
tcaaactgcggatcatcacgt

SEQ ID NO: 7 - DNA, 19 bp, synthetic construct
  misc_feature 1..19: note = BVDV specific forward primer
  source 1..19: mol_type = other DNA
tgacaccatcaccgaccac

SEQ ID NO: 8 - DNA, 21 bp, synthetic construct
  misc_feature 1..21: note = BVDV specific reverse primer
  source 1..21: mol_type = other DNA
ctccctctctgcccatttctt

SEQ ID NO: 9 - DNA, 23 bp, synthetic construct
  misc_feature 1..23: note = BRV specific forward primer
  source 1..23: mol_type = other DNA
tcatttcagttgatgagaccacc

SEQ ID NO: 10 - DNA, 25 bp, synthetic construct
  misc_feature 1..25: note = BRV specific reverse primer
  source 1..25: mol_type = other DNA
attcaattctaagcgtgagtcctac

SEQ ID NO: 11 - DNA, 27 bp, synthetic construct
  misc_feature 1..27: note = CPV specific forward primer
  source 1..27: mol_type = other DNA
agctagtttcatcttaactatcaaatt

SEQ ID NO: 12 - DNA, 23 bp, synthetic construct
  misc_feature 1..23: note = CPV specific reverse primer
  source 1..23: mol_type = other DNA
ttaactctccagaaaactcatgc